European Patent Application EP 4 467 572 A1, published November 27, 2024. Title: 改変された組換えアデノ随伴ウイルス（ＡＡＶ）結合性タンパク質及び感染能に基づくＡＡＶの分析方法. Applicant: 東ソー株式会社. Application JP. The sequence listing filed with the application follows.

SEQUENCE LISTING (103 sequences)

SEQ ID NO: 1 - protein, 1049 aa, Homo sapiens
MEKRLGVKPNPASWILSGYYWQTSAKWLRSLYLFYTCFCFSVLWLSTDASESRCQQGKTQFGVGLRSGGENHLWLLEGTPSLQSCWAACCQDSACHVFWWLEGMCIQADCSRPQSCRAFRTHSSNSMLVFLKKFQTADDLGFLPEDDVPHLLGLGWNWASWRQSPPRAALRPAVSSSDQQSLIRKLQKRGSPSDVVTPIVTQHSKVNDSNELGGLTTSGSAEVHKAITISSPLTTDLTAELSGGPKNVSVQPEISEGLATTPSTQQVKSSEKTQIAVPQPVAPSYSYATPTPQASFQSTSAPYPVIKELVVSAGESVQITLPKNEVQLNAYVLQEPPKGETYTYDWQLITHPRDYSGEMEGKHSQILKLSKLTPGLYEFKVIVEGQNAHGEGYVNVTVKPEPRKNRPPIAIVSPQFQEISLPTTSTVIDGSQSTDDDKIVQYHWEELKGPLREEKISEDTAILKLSKLVPGNYTFSLTVVDSDGATNSTTANLTVNKAVDYPPVANAGPNQVITLPQNSITLFGNQSTDDHGITSYEWSLSPSSKGKVVEMQGVRTPTLQLSAMQEGDYTYQLTVTDTIGQQATAQVTVIVQPENNKPPQADAGPDKELTLPVDSTTLDGSKSSDDQKIISYLWEKTQGPDGVQLENANSSVATVTGLQVGTYVFTLTVKDERNLQSQSSVNVIVKEEINKPPIAKITGNVVITLPTSTAELDGSKSSDDKGIVSYLWTRDEGSPAAGEVLNHSDHHPILFLSNLVEGTYTFHLKVTDAKGESDTDRTTVEVKPDPRKNNLVEIILDINVSQLTERLKGMFIRQIGVLLGVLDSDIIVQKIQPYTEQSTKMVFFVQNEPPHQIFKGHEVAAMLKSELRKQKADFLIFRALEVNTVTCQLNCSDHGHCDSFTKRCICDPFWMENFIKVQLRDGDSNCEWSVLYVIIATFVIVVALGILSWTVICCCKRQKGKPKRKSKYKILDATDQESLELKPTSRAGIKQKGLLLSSSLMHSESELDSDDAIFTWPDREKGKLLHGQNGSVPNGQTPLKARSPREEIL

SEQ ID NO: 2 - protein, 239 aa, synthetic construct
  REGION 1..239: note = EGFP protein
MVSKGEELFTGVVPILVELDGDVNGHKFSVSGEGEGDATYGKLTLKFICTTGKLPVPWPTLVTTLTYGVQCFSRYPDHMKQHDFFKSAMPEGYVQERTIFFKDDGNYKTRAEVKFEGDTLVNRIELKGIDFKEDGNILGHKLEYNYNSHNVYIMADKQKNGIKVNFKIRHNIEDGSVQLADHYQQNTPIGDGPVLLPDNHYLSTQSALSKDPNEKRDHMVLLEFVTAAGITLGMDELYK

SEQ ID NO: 3 - DNA, 732 bp, synthetic construct
  misc_feature 1..732: note = EGFP gene
  source 1..732: mol_type = other DNA
gaattcatggtgagcaaaggcgaggaactgtttactggtgtagtccccatactggtggaacttgatggggatgtcaatggtcacaaatttagcgtgtcaggagaaggcgaaggagatgcgacgtacggcaagctgacccttaagttcatctgtaccacgggtaagttgcctgttccttggcccacacttgtgacaaccctgacctatggagtgcaatgcttctccagatatccagaccacatgaagcagcatgacttcttcaaatccgccatgccagaaggctatgtgcaggaaaggaccatcttctttaaggacgacggaaactacaaaactcgtgctgaggtgaagttcgaaggagacacactggtgaatcgaatcgagctgaaagggattgactttaaggaggacgggaatattctgggccataagctggagtacaactacaactctcacaatgtgtacatcatggccgacaaacagaagaacgggattaaggtcaactttaagattcgccacaacatcgaggatggtagtgtacagctcgctgaccattaccagcagaatactcccataggcgatggaccagttttgctgcctgacaaccattatctgtcaacccaatctgccctgagcaaagatccgaatgagaaacgggatcacatggttctcttggagtttgtcacagcagcagggatcactctcggcatggatgagctctataaatagggatcc

SEQ ID NO: 4 - protein, 219 aa, synthetic construct
  REGION 1..219: note = AVR10s
MKYLLPTAAAGLLLLAAQPAMAMGSAGESDQITLPKNEVQLNAYVLQEPPKGETSTYDWQLITHPRDYSGEMEGEHSQILKLSNLTPGLYEFKAVVEGQNAHSEGYVNVTVEPEPRKNRPPIAIVSPQFQEISLPTTSTVIDGSQSTDDDKIVQYHWEELKGPLREEKISEDTAILKLSKLVPGNYTFRLTVVDSDGATDSTTANLTVNKAVDHHHHHH

SEQ ID NO: 5 - DNA, 30 bp, synthetic construct
  misc_feature 1..30: note = Primer A330X-F
  misc_feature 18..19: note = n is a, c, g, or t
  source 1..30: mol_type = other DNA
ttttggtctcactgaatnnktatgtgctgc

SEQ ID NO: 6 - DNA, 31 bp, synthetic construct
  misc_feature 1..31: note = Primer A330X-R
  source 1..31: mol_type = other DNA
ttttggtctcatcagttgtacttcgttcttc

SEQ ID NO: 7 - DNA, 30 bp, synthetic construct
  misc_feature 1..30: note = Primer Y331X-F
  misc_feature 21..22: note = n is a, c, g, or t
  source 1..30: mol_type = other DNA
ttttggtctcactgaatgcgnnkgtgctgc

SEQ ID NO: 8 - DNA, 31 bp, synthetic construct; identical to SEQ ID NO: 6
  misc_feature 1..31: note = Primer Y331X-R
  source 1..31: mol_type = other DNA

SEQ ID NO: 9 - DNA, 34 bp, synthetic construct
  misc_feature 1..34: note = Primer V332X-F
  misc_feature 22..23: note = n is a, c, g, or t
  source 1..34: mol_type = other DNA
ttttggtctcagaatgcgtatnnkctgcaggaac

SEQ ID NO: 10 - DNA, 33 bp, synthetic construct
  misc_feature 1..33: note = Primer V332X-R
  source 1..33: mol_type = other DNA
ttttggtctcaattcagttgtacttcgttcttc

SEQ ID NO: 11 - DNA, 34 bp, synthetic construct
  misc_feature 1..34: note = Primer L333X-F
  misc_feature 25..26: note = n is a, c, g, or t
  source 1..34: mol_type = other DNA
ttttggtctcagaatgcgtatgtgnnkcaggaac

SEQ ID NO: 12 - DNA, 33 bp, synthetic construct; identical to SEQ ID NO: 10
  misc_feature 1..33: note = Primer L333X-R
  source 1..33: mol_type = other DNA

SEQ ID NO: 13 - DNA, 20 bp, synthetic construct
  misc_feature 1..20: note = Forward primer
  source 1..20: mol_type = other DNA
taatacgactcactataggg

SEQ ID NO: 14 - DNA, 21 bp, synthetic construct
  misc_feature 1..21: note = Reverse primer
  source 1..21: mol_type = other DNA
atgctagttattgctcagcgg

SEQ ID NO: 15 - protein, 219 aa, synthetic construct
  REGION 1..219: note = AVR10s_A330C
MKYLLPTAAAGLLLLAAQPAMAMGSAGESDQITLPKNEVQLNCYVLQEPPKGETSTYDWQLITHPRDYSGEMEGEHSQILKLSNLTPGLYEFKAVVEGQNAHSEGYVNVTVEPEPRKNRPPIAIVSPQFQEISLPTTSTVIDGSQSTDDDKIVQYHWEELKGPLREEKISEDTAILKLSKLVPGNYTFRLTVVDSDGATDSTTANLTVNKAVDHHHHHH

SEQ ID NO: 16 - protein, 219 aa, synthetic construct
  REGION 1..219: note = AVR10s_A330F
MKYLLPTAAAGLLLLAAQPAMAMGSAGESDQITLPKNEVQLNFYVLQEPPKGETSTYDWQLITHPRDYSGEMEGEHSQILKLSNLTPGLYEFKAVVEGQNAHSEGYVNVTVEPEPRKNRPPIAIVSPQFQEISLPTTSTVIDGSQSTDDDKIVQYHWEELKGPLREEKISEDTAILKLSKLVPGNYTFRLTVVDSDGATDSTTANLTVNKAVDHHHHHH

SEQ ID NO: 17 - protein, 219 aa, synthetic construct
  REGION 1..219: note = AVR10s_A330L
MKYLLPTAAAGLLLLAAQPAMAMGSAGESDQITLPKNEVQLNLYVLQEPPKGETSTYDWQLITHPRDYSGEMEGEHSQILKLSNLTPGLYEFKAVVEGQNAHSEGYVNVTVEPEPRKNRPPIAIVSPQFQEISLPTTSTVIDGSQSTDDDKIVQYHWEELKGPLREEKISEDTAILKLSKLVPGNYTFRLTVVDSDGATDSTTANLTVNKAVDHHHHHH

SEQ ID NO: 18 - protein, 219 aa, synthetic construct
  REGION 1..219: note = AVR10s_A330R
MKYLLPTAAAGLLLLAAQPAMAMGSAGESDQITLPKNEVQLNRYVLQEPPKGETSTYDWQLITHPRDYSGEMEGEHSQILKLSNLTPGLYEFKAVVEGQNAHSEGYVNVTVEPEPRKNRPPIAIVSPQFQEISLPTTSTVIDGSQSTDDDKIVQYHWEELKGPLREEKISEDTAILKLSKLVPGNYTFRLTVVDSDGATDSTTANLTVNKAVDHHHHHH

SEQ ID NO: 19 - protein, 219 aa, synthetic construct
  REGION 1..219: note = AVR10s_A330V (AVR11a)
MKYLLPTAAAGLLLLAAQPAMAMGSAGESDQITLPKNEVQLNVYVLQEPPKGETSTYDWQLITHPRDYSGEMEGEHSQILKLSNLTPGLYEFKAVVEGQNAHSEGYVNVTVEPEPRKNRPPIAIVSPQFQEISLPTTSTVIDGSQSTDDDKIVQYHWEELKGPLREEKISEDTAILKLSKLVPGNYTFRLTVVDSDGATDSTTANLTVNKAVDHHHHHH

SEQ ID NO: 20 - protein, 219 aa, synthetic construct
  REGION 1..219: note = AVR10s_A330W
MKYLLPTAAAGLLLLAAQPAMAMGSAGESDQITLPKNEVQLNWYVLQEPPKGETSTYDWQLITHPRDYSGEMEGEHSQILKLSNLTPGLYEFKAVVEGQNAHSEGYVNVTVEPEPRKNRPPIAIVSPQFQEISLPTTSTVIDGSQSTDDDKIVQYHWEELKGPLREEKISEDTAILKLSKLVPGNYTFRLTVVDSDGATDSTTANLTVNKAVDHHHHHH

SEQ ID NO: 21 - protein, 219 aa, synthetic construct
  REGION 1..219: note = AVR10s_A330Y
MKYLLPTAAAGLLLLAAQPAMAMGSAGESDQITLPKNEVQLNYYVLQEPPKGETSTYDWQLITHPRDYSGEMEGEHSQILKLSNLTPGLYEFKAVVEGQNAHSEGYVNVTVEPEPRKNRPPIAIVSPQFQEISLPTTSTVIDGSQSTDDDKIVQYHWEELKGPLREEKISEDTAILKLSKLVPGNYTFRLTVVDSDGATDSTTANLTVNKAVDHHHHHH

SEQ ID NO: 22 - protein, 219 aa, synthetic construct
  REGION 1..219: note = AVR10s_Y331C
MKYLLPTAAAGLLLLAAQPAMAMGSAGESDQITLPKNEVQLNACVLQEPPKGETSTYDWQLITHPRDYSGEMEGEHSQILKLSNLTPGLYEFKAVVEGQNAHSEGYVNVTVEPEPRKNRPPIAIVSPQFQEISLPTTSTVIDGSQSTDDDKIVQYHWEELKGPLREEKISEDTAILKLSKLVPGNYTFRLTVVDSDGATDSTTANLTVNKAVDHHHHHH

SEQ ID NO: 23 - protein, 219 aa, synthetic construct
  REGION 1..219: note = AVR10s_V332W
MKYLLPTAAAGLLLLAAQPAMAMGSAGESDQITLPKNEVQLNAYWLQEPPKGETSTYDWQLITHPRDYSGEMEGEHSQILKLSNLTPGLYEFKAVVEGQNAHSEGYVNVTVEPEPRKNRPPIAIVSPQFQEISLPTTSTVIDGSQSTDDDKIVQYHWEELKGPLREEKISEDTAILKLSKLVPGNYTFRLTVVDSDGATDSTTANLTVNKAVDHHHHHH

SEQ ID NO: 24 - protein, 219 aa, synthetic construct
  REGION 1..219: note = AVR10s_V332Y
MKYLLPTAAAGLLLLAAQPAMAMGSAGESDQITLPKNEVQLNAYYLQEPPKGETSTYDWQLITHPRDYSGEMEGEHSQILKLSNLTPGLYEFKAVVEGQNAHSEGYVNVTVEPEPRKNRPPIAIVSPQFQEISLPTTSTVIDGSQSTDDDKIVQYHWEELKGPLREEKISEDTAILKLSKLVPGNYTFRLTVVDSDGATDSTTANLTVNKAVDHHHHHH

SEQ ID NO: 25 - protein, 219 aa, synthetic construct
  REGION 1..219: note = AVR10s_L333C
MKYLLPTAAAGLLLLAAQPAMAMGSAGESDQITLPKNEVQLNAYVCQEPPKGETSTYDWQLITHPRDYSGEMEGEHSQILKLSNLTPGLYEFKAVVEGQNAHSEGYVNVTVEPEPRKNRPPIAIVSPQFQEISLPTTSTVIDGSQSTDDDKIVQYHWEELKGPLREEKISEDTAILKLSKLVPGNYTFRLTVVDSDGATDSTTANLTVNKAVDHHHHHH

SEQ ID NO: 26 - DNA, 38 bp, synthetic construct
  source 1..38: mol_type = other DNA
  misc_feature 1..38: note = Primer Q347X-F
ttttggtctcagtatgactggnnkcttattacgcatcc

SEQ ID NO: 27 - DNA, 35 bp, synthetic construct
  source 1..35: mol_type = other DNA
  misc_feature 1..35: note = Primer Q347X-R
ttttggtctcaatacgtcgaggtttcccctttcgg

SEQ ID NO: 28 - DNA, 38 bp, synthetic construct
  source 1..38: mol_type = other DNA
  misc_feature 1..38: note = Primer L348X-F
ttttggtctcagtatgactggcagnnkattacgcatcc

SEQ ID NO: 29 - DNA, 35 bp, synthetic construct; identical to SEQ ID NO: 27
  source 1..35: mol_type = other DNA
  misc_feature 1..35: note = Primer L348X-R

SEQ ID NO: 30 - DNA, 38 bp, synthetic construct
  source 1..38: mol_type = other DNA
  misc_feature 1..38: note = Primer I349X-F
ttttggtctcagtatgactggcagcttnnkacgcatcc

SEQ ID NO: 31 - DNA, 35 bp, synthetic construct; identical to SEQ ID NO: 27
  source 1..35: mol_type = other DNA
  misc_feature 1..35: note = Primer I349X-R

SEQ ID NO: 32 - protein, 219 aa, synthetic construct
  REGION 1..219: note = AVR10s_Q347S
MKYLLPTAAAGLLLLAAQPAMAMGSAGESDQITLPKNEVQLNAYVLQEPPKGETSTYDWSLITHPRDYSGEMEGEHSQILKLSNLTPGLYEFKAVVEGQNAHSEGYVNVTVEPEPRKNRPPIAIVSPQFQEISLPTTSTVIDGSQSTDDDKIVQYHWEELKGPLREEKISEDTAILKLSKLVPGNYTFRLTVVDSDGATDSTTANLTVNKAVDHHHHHH

SEQ ID NO: 33 - protein, 219 aa, synthetic construct
  REGION 1..219: note = AVR10s_L348C
MKYLLPTAAAGLLLLAAQPAMAMGSAGESDQITLPKNEVQLNAYVLQEPPKGETSTYDWQCITHPRDYSGEMEGEHSQILKLSNLTPGLYEFKAVVEGQNAHSEGYVNVTVEPEPRKNRPPIAIVSPQFQEISLPTTSTVIDGSQSTDDDKIVQYHWEELKGPLREEKISEDTAILKLSKLVPGNYTFRLTVVDSDGATDSTTANLTVNKAVDHHHHHH

SEQ ID NO: 34 - protein, 219 aa, synthetic construct
  REGION 1..219: note = AVR10s_I349N
MKYLLPTAAAGLLLLAAQPAMAMGSAGESDQITLPKNEVQLNAYVLQEPPKGETSTYDWQLNTHPRDYSGEMEGEHSQILKLSNLTPGLYEFKAVVEGQNAHSEGYVNVTVEPEPRKNRPPIAIVSPQFQEISLPTTSTVIDGSQSTDDDKIVQYHWEELKGPLREEKISEDTAILKLSKLVPGNYTFRLTVVDSDGATDSTTANLTVNKAVDHHHHHH

SEQ ID NO: 35 - DNA, 657 bp, synthetic construct
  source 1..657: mol_type = other DNA
  misc_feature 1..657: note = AVR10s_A330V (AVR11a) gene
atgaaatacctgctgccgaccgctgctgctggtctgctgctcctcgctgcccagccggcgatggccatgggctctgcaggcgagtcggatcagattaccctgccgaagcacgaagcacaactgaatgtttatgtgctgctggtaccaccgaaaggggaagcctcgacgtatgactggcagcttattacgcatcctcgcgactacagcggcgagatggaaggagaacattcgcagattctgaaactgtccaatctgacgccgggtctgtatgaataccgtgctgtcgttgaaggtcagaatgcacatagcgaaggctatgttaacgttaccgtggaaccggagccacgcaagaaccgtcctccgatcgccattgtttcaccgcagtttcaggagatttcactgccgaccaccagtaccgttatcgatggttcgcagtcaacggatgacgacaaaatcgttcagtaccactgggaagagctgaaaggccccttacgcgaagagaagatcagcgaagataccgccatcttgaaattatcgcagcttgtgccgggtaactacacgttcagactgacggtggtcgataccgatggcgcaaccgactccaccaccgccgatcttaccgtcaacaaagcggtagaccatcatcatcatcatcat

SEQ ID NO: 36 - DNA, 657 bp, synthetic construct
  source 1..657: mol_type = other DNA
  misc_feature 1..657: note = AVR11a_Q334L gene
atgaaatacctgctgccgaccgctgctgctggtctgctgctcctcgctgcccagccggcgatggccatgggctctgcaggcgagtcggatcagattaccctgccgaagaacgaagtacaactgaatgtttatgtgctgctggaaccaccgaaaggggaaacctcgacgtatgactggcagcttattacgcatcctcgcgactacagcggcgagatggaaggagaacattcgcagattctgaaactgtccaatctgacgccgggtctgtatgaattcaaggctgtcgttgaaggtcagaatgcacatagcgaaggctatgttaacgttaccgtggaaccggagccacgcaagaaccgtcctccgatcgccattgtttcaccgcagttccaggagatttcactgccgaccaccagtaccgttatcgatggttcgcagtcaacggatgacgacaaaatcgttcagtaccactgggaagagctgaaaggccccttacgcgaagagaagatcagcgaagataccgccatcttgaaattatcgaaacttgtgccgggtaactacacgttcagactgacggtagtcgattctgatggcgcaaccgactccaccaccgccaaccttaccgtcaacaaagcggtagaccatcatcatcatcatcat

SEQ ID NO: 37 - protein, 219 aa, synthetic construct
  REGION 1..219: note = AVR11a_Q334L
MKYLLPTAAAGLLLLAAQPAMAMGSAGESDQITLPKNEVQLNVYVLLEPPKGETSTYDWQLITHPRDYSGEMEGEHSQILKLSNLTPGLYEFKAVVEGQNAHSEGYVNVTVEPEPRKNRPPIAIVSPQFQEISLPTTSTVIDGSQSTDDDKIVQYHWEELKGPLREEKISEDTAILKLSKLVPGNYTFRLTVVDSDGATDSTTANLTVNKAVDHHHHHH

SEQ ID NO: 38 - DNA, 657 bp, synthetic construct
  source 1..657: mol_type = other DNA
  misc_feature 1..657: note = AVR11a_T341A gene
atgaaatacctgctgccgaccgctgctgctggtctgctgctcctcgctgcccagccggcgatggccatgggctctgcaggcgagtcggatcagattaccctgccgaagaacgaagtacaactgaatgtttatgtgctgcaggaaccaccgaaaggggaagcctcgacgtatgactggcagcttattacgcatcctcgcgactacagcggcgagatggaaggagaacattcgcagattctgaaactgtccaatctgacgccgggtctgtatgaattcaaggctgtcgttgaaggtcagaatgcacatagcgaaggctatgttaacgttaccgtggaaccggagccacgcaagaaccgtcctccgatcgccattgtttcaccgcagtttcaggagatttcactgccgaccaccagtaccgttatcgatggttcgcagtcaacggatgacgacaaaatcgttcagtaccactgggaagagctgaaaggccccttacgcgaagagaagatcagcgaagataccgccatcttgaaattatcgaaacttgtgccgggtaactacacgttcagactgacggtggtcgattctgatggcgcaaccgactccaccaccgccaaccttaccgtcaacaaagcggtagaccatcatcatcatcatcat

SEQ ID NO: 39 - protein, 219 aa, synthetic construct
  REGION 1..219: note = AVR11a_T341A
MKYLLPTAAAGLLLLAAQPAMAMGSAGESDQITLPKNEVQLNVYVLLEPPKGEASTYDWQLITHPRDYSGEMEGEHSQILKLSNLTPGLYEFKAVVEGQNAHSEGYVNVTVEPEPRKNRPPIAIVSPQFQEISLPTTSTVIDGSQSTDDDKIVQYHWEELKGPLREEKISEDTAILKLSKLVPGNYTFRLTVVDSDGATDSTTANLTVNKAVDHHHHHH

SEQ ID NO: 40 - DNA, 657 bp, synthetic construct
  source 1..657: mol_type = other DNA
  misc_feature 1..657: note = AVR11a_M359I gene
atgaaatacctgctgccgaccgctgctgctggtctgctgctcctcgctgcccagccggcgatggccatgggctctgcaggcgagtcggatcagattaccctgccgaagaacgaagtacaactgaatgtttatgtgctgcaggaaccaccgaaaggggaaacctcgacgtatgactggcagcttattacgcatcctcgcgactacagcggcgagatagaaggagaacattcgcagattctgaaactgtccaatctgacgccgggtctgtatgaattcaaggctgtcgttgaaggtcagaatgcacatagcgaaggctatgttaacgttaccgtggaaccggagccacgcaagaaccgtcctccgatcgccattgtttcaccgcagtttcaggagatttcactgccgaccaccagtaccgttatcgatggttcgcagtcaacggatgacgacaaaatcgttcagtaccactgggaagagctgaaaggccccttacgcgaagagaagatcagcgaagataccgccatcttgaaattatcgaaacttgtgccgggtaactacacgttcagactgacggtggtcgattctgatggcgcaaccgactccaccaccgccaaccttaccgtcaacaaagcggtagaccatcatcatcatcatcat

SEQ ID NO: 41 - protein, 219 aa, synthetic construct
  REGION 1..219: note = AVR11a_M359I
MKYLLPTAAAGLLLLAAQPAMAMGSAGESDQITLPKNEVQLNVYVLQEPPKGETSTYDWQLITHPRDYSGEIEGEHSQILKLSNLTPGLYEFKAVVEGQNAHSEGYVNVTVEPEPRKNRPPIAIVSPQFQEISLPTTSTVIDGSQSTDDDKIVQYHWEELKGPLREEKISEDTAILKLSKLVPGNYTFRLTVVDSDGATDSTTANLTVNKAVDHHHHHH

SEQ ID NO: 42 - DNA, 657 bp, synthetic construct
  source 1..657: mol_type = other DNA
  misc_feature 1..657: note = AVR11a_F379Y gene
atgaaatacctgctgccgaccgctgctgctggtctgctgctcctcgctgcccagccggcgatggccatgggctctgcaggcgagtcggatcagattaccctgccgaagaacgaagtacaactgaatgtttatgtgctgcaggaaccaccgaaaggggaaacctcgacgtatgactggcagcttattacgcatcctcgcgactacagcggcgagatggaaggagaacattcgcagattctgaaactgtccaatctgacgccgggtctgtatgaatacaaggctgtcgttgaaggtcagaatgcacatagcgaaggctatgttaacgttaccgtggaaccggagccacgcaagaaccgtcctccgatcgccattgtttcaccgcagtttcaggagatttcactgccgaccaccagtaccgttatcgatggttcgcagtcaacggatgacgacaaaatcgttcagtaccactgggaagagctgaaaggccccttacgcgaagagaagatcagcgaagataccgccatcttgaaattatcgaaacttgtgccgggtaactacacgttcagactgacggtggtcgattctgatggcgcaaccgactccaccaccgccaaccttaccgtcaacaaagcggtagaccatcatcatcatcatcat

SEQ ID NO: 43 - protein, 219 aa, synthetic construct
  REGION 1..219: note = AVR11a_F379Y
MKYLLPTAAAGLLLLAAQPAMAMGSAGESDQITLPKNEVQLNVYVLQEPPKGETSTYDWQLITHPRDYSGEMEGEHSQILKLSNLTPGLYEYKAVVEGQNAHSEGYVNVTVEPEPRKNRPPIAIVSPQFQEISLPTTSTVIDGSQSTDDDKIVQYHWEELKGPLREEKISEDTAILKLSKLVPGNYTFRLTVVDSDGATDSTTANLTVNKAVDHHHHHH

SEQ ID NO: 44 - DNA, 39 bp, synthetic construct
  source 1..39: mol_type = other DNA
  misc_feature 1..39: note = Primer N324H-F
ttttggtctcacattcagttgtacttcgtgcttcggcag

SEQ ID NO: 45 - DNA, 42 bp, synthetic construct
  source 1..42: mol_type = other DNA
  misc_feature 1..42: note = Primer N324H-R
ttttggtctcaaatgtttatgtgctgcaggaaccaccgaaag

SEQ ID NO: 46 - DNA, 39 bp, synthetic construct
  source 1..39: mol_type = other DNA
  misc_feature 1..39: note = Primer E335V-F
ttttggtctcacattcagttgtacttcgttcttcggcag

SEQ ID NO: 47 - DNA, 42 bp, synthetic construct
  source 1..42: mol_type = other DNA
  misc_feature 1..42: note = Primer E335V-R
ttttggtctcaaatgtttatgtgctgcaggtaccaccgaaag

SEQ ID NO: 48 - DNA, 39 bp, synthetic construct; identical to SEQ ID NO: 44
  source 1..39: mol_type = other DNA
  misc_feature 1..39: note = Primer N324H+E335V-F

SEQ ID NO: 49 - DNA, 42 bp, synthetic construct; identical to SEQ ID NO: 47
  source 1..42: mol_type = other DNA
  misc_feature 1..42: note = Primer N324H+E335V-R

SEQ ID NO: 50 - DNA, 39 bp, synthetic construct; identical to SEQ ID NO: 44
  source 1..39: mol_type = other DNA
  misc_feature 1..39: note = Primer N324H+Q334L+E335V-F

SEQ ID NO: 51 - DNA, 42 bp, synthetic construct
  source 1..42: mol_type = other DNA
  misc_feature 1..42: note = Primer N324H+Q334L+E335V-R
ttttggtctcaaatgtttatgtgctgctggtaccaccgaaag

SEQ ID NO: 52 - DNA, 38 bp, synthetic construct
  source 1..38: mol_type = other DNA
  misc_feature 1..38: note = Primer T341A-F
ttttggtctcatttcggtggtaccagcagcacataaac

SEQ ID NO: 53 - DNA, 34 bp, synthetic construct
  source 1..34: mol_type = other DNA
  misc_feature 1..34: note = Primer T341A-R
ttttggtctcagaaaggggaagcctcgacgtatg

SEQ ID NO: 54 - protein, 219 aa, synthetic construct
  REGION 1..219: note = AVR12a
MKYLLPTAAAGLLLLAAQPAMAMGSAGESDQITLPKHEVQLNVYVLQEPPKGETSTYDWQLITHPRDYSGEMEGEHSQILKLSNLTPGLYEFKAVVEGQNAHSEGYVNVTVEPEPRKNRPPIAIVSPQFQEISLPTTSTVIDGSQSTDDDKIVQYHWEELKGPLREEKISEDTAILKLSKLVPGNYTFRLTVVDSDGATDSTTANLTVNKAVDHHHHHH

SEQ ID NO: 55 - protein, 219 aa, synthetic construct
  REGION 1..219: note = AVR12b
MKYLLPTAAAGLLLLAAQPAMAMGSAGESDQITLPKNEVQLNVYVLQVPPKGETSTYDWQLITHPRDYSGEMEGEHSQILKLSNLTPGLYEFKAVVEGQNAHSEGYVNVTVEPEPRKNRPPIAIVSPQFQEISLPTTSTVIDGSQSTDDDKIVQYHWEELKGPLREEKISEDTAILKLSKLVPGNYTFRLTVVDSDGATDSTTANLTVNKAVDHHHHHH

SEQ ID NO: 56 - protein, 219 aa, synthetic construct
  REGION 1..219: note = AVR13
MKYLLPTAAAGLLLLAAQPAMAMGSAGESDQITLPKHEVQLNVYVLQVPPKGETSTYDWQLITHPRDYSGEMEGEHSQILKLSNLTPGLYEFKAVVEGQNAHSEGYVNVTVEPEPRKNRPPIAIVSPQFQEISLPTTSTVIDGSQSTDDDKIVQYHWEELKGPLREEKISEDTAILKLSKLVPGNYTFRLTVVDSDGATDSTTANLTVNKAVDHHHHHH

SEQ ID NO: 57 - protein, 219 aa, synthetic construct
  REGION 1..219: note = AVR14a
MKYLLPTAAAGLLLLAAQPAMAMGSAGESDQITLPKHEVQLNVYVLQVPPKGEASTYDWQLITHPRDYSGEMEGEHSQILKLSNLTPGLYEFKAVVEGQNAHSEGYVNVTVEPEPRKNRPPIAIVSPQFQEISLPTTSTVIDGSQSTDDDKIVQYHWEELKGPLREEKISEDTAILKLSKLVPGNYTFRLTVVDSDGATDSTTANLTVNKAVDHHHHHH

SEQ ID NO: 58 - protein, 219 aa, synthetic construct
  REGION 1..219: note = AVR14b
MKYLLPTAAAGLLLLAAQPAMAMGSAGESDQITLPKHEVQLNVYVLLVPPKGETSTYDWQLITHPRDYSGEMEGEHSQILKLSNLTPGLYEFKAVVEGQNAHSEGYVNVTVEPEPRKNRPPIAIVSPQFQEISLPTTSTVIDGSQSTDDDKIVQYHWEELKGPLREEKISEDTAILKLSKLVPGNYTFRLTVVDSDGATDSTTANLTVNKAVDHHHHHH

SEQ ID NO: 59 - protein, 219 aa, synthetic construct
  REGION 1..219: note = AVR14c
MKYLLPTAAAGLLLLAAQPAMAMGSAGESDQITLPKHEVQLNVYVLQVPPKGETSTYDWQLITHPRDYSGEIEGEHSQILKLSNLTPGLYEFKAVVEGQNAHSEGYVNVTVEPEPRKNRPPIAIVSPQFQEISLPTTSTVIDGSQSTDDDKIVQYHWEELKGPLREEKISEDTAILKLSKLVPGNYTFRLTVVDSDGATDSTTANLTVNKAVDHHHHHH

SEQ ID NO: 60 - protein, 219 aa, synthetic construct
  REGION 1..219: note = AVR14d
MKYLLPTAAAGLLLLAAQPAMAMGSAGESDQITLPKHEVQLNVYVLQVPPKGETSTYDWQLITHPRDYSGEMEGEHSQILKLSNLTPGLYEYKAVVEGQNAHSEGYVNVTVEPEPRKNRPPIAIVSPQFQEISLPTTSTVIDGSQSTDDDKIVQYHWEELKGPLREEKISEDTAILKLSKLVPGNYTFRLTVVDSDGATDSTTANLTVNKAVDHHHHHH

SEQ ID NO: 61 - protein, 219 aa, synthetic construct
  REGION 1..219: note = AVR15a
MKYLLPTAAAGLLLLAAQPAMAMGSAGESDQITLPKHEVQLNVYVLLVPPKGEASTYDWQLITHPRDYSGEMEGEHSQILKLSNLTPGLYEFKAVVEGQNAHSEGYVNVTVEPEPRKNRPPIAIVSPQFQEISLPTTSTVIDGSQSTDDDKIVQYHWEELKGPLREEKISEDTAILKLSKLVPGNYTFRLTVVDSDGATDSTTANLTVNKAVDHHHHHH

SEQ ID NO: 62 - protein, 219 aa, synthetic construct
  REGION 1..219: note = AVR15b
MKYLLPTAAAGLLLLAAQPAMAMGSAGESDQITLPKHEVQLNVYVLLVPPKGETSTYDWQLITHPRDYSGEIEGEHSQILKLSNLTPGLYEFKAVVEGQNAHSEGYVNVTVEPEPRKNRPPIAIVSPQFQEISLPTTSTVIDGSQSTDDDKIVQYHWEELKGPLREEKISEDTAILKLSKLVPGNYTFRLTVVDSDGATDSTTANLTVNKAVDHHHHHH

SEQ ID NO: 63 - protein, 219 aa, synthetic construct
  REGION 1..219: note = AVR15c
MKYLLPTAAAGLLLLAAQPAMAMGSAGESDQITLPKHEVQLNVYVLLVPPKGETSTYDWQLITHPRDYSGEMEGEHSQILKLSNLTPGLYEYKAVVEGQNAHSEGYVNVTVEPEPRKNRPPIAIVSPQFQEISLPTTSTVIDGSQSTDDDKIVQYHWEELKGPLREEKISEDTAILKLSKLVPGNYTFRLTVVDSDGATDSTTANLTVNKAVDHHHHHH

SEQ ID NO: 64 - DNA, 657 bp, synthetic construct
  source 1..657: mol_type = other DNA
  misc_feature 1..657: note = AVR15c gene
atgaaatacctgctgccgaccgctgctgctggtctgctgctcctcgctgcccagccggcgatggccatgggctctgcaggcgagtcggatcagattaccctgccgaagcacgaagtacaactgaatgtttatgtgctgctggtaccaccgaaaggggaaacctcgacgtatgactggcagcttattacgcatcctcgcgactacagcggcgagatggaaggagaacattcgcagattctgaaactgtccaatctgacgccgggtctgtatgaatacaaggctgtcgttgaaggtcagaatgcacatagcgaaggctatgttaacgttaccgtggaaccggagccacgcaagaaccgtcctccgatcgccattgtttcaccgcagtttcaggagatttcactgccgaccaccagtaccgttatcgatggttcgcagtcaacggatgacgacaaaatcgttcagtaccactgggaagagctgaaaggccccttacgcgaagagaagatcagcgaagataccgccatcttgaaattatcgaaacttgtgccgggtaactacacgttcagactgacggtggtcgattctgatggcgcaaccgactccaccaccgccaaccttaccgtcaacaaagcggtagaccatcatcatcatcatcat

SEQ ID NO: 65 - protein, 219 aa, synthetic construct
  REGION 1..219: note = AVR16
MKYLLPTAAAGLLLLAAQPAMAMGSAGESDQITLPKHEVQLNVYVLLVPPKGEASTYDWQLITHPRDYSGEMEGEHSQILKLSNLTPGLYEYKAVVEGQNAHSEGYVNVTVEPEPRKNRPPIAIVSPQFQEISLPTTSTVIDGSQSTDDDKIVQYHWEELKGPLREEKISEDTAILKLSKLVPGNYTFRLTVVDSDGATDSTTANLTVNKAVDHHHHHH

SEQ ID NO: 66 - DNA, 657 bp, synthetic construct
  source 1..657: mol_type = other DNA
  misc_feature 1..657: note = AVR16 gene
atgaaatacctgctgccgaccgctgctgctggtctgctgctcctcgctgcccagccggcgatggccatgggctctgcaggcgagtcggatcagattaccctgccgaagcacgaagtacaactgaatgtttatgtgctgctggtaccaccgaaaggggaagcctcgacgtatgactggcagcttattacgcatcctcgcgactacagcggcgagatggaaggagaacattcgcagattctgaaactgtccaatctgacgccgggtctgtatgaatacaaggctgtcgttgaaggtcagaatgcacatagcgaaggctatgttaacgttaccgtggaaccggagccacgcaagaaccgtcctccgatcgccattgtttcaccgcagtttcaggagatttcactgccgaccaccagtaccgttatcgatggttcgcagtcaacggatgacgacaaaatcgttcagtaccactgggaagagctgaaaggccccttacgcgaagagaagatcagcgaagataccgccatcttgaaattatcgaaacttgtgccgggtaactacacgttcagactgacggtggtcgattctgatggcgcaaccgactccaccaccgccaaccttaccgtcaacaaagcggtagaccatcatcatcatcatcat

SEQ ID NO: 67 - protein, 219 aa, synthetic construct
  REGION 1..219: note = AVR16_V326A
MKYLLPTAAAGLLLLAAQPAMAMGSAGESDQITLPKHEAQLNVYVLLVPPKGEASTYDWQLITHPRDYSGEMEGEHSQILKLSNLTPGLYEYKAVVEGQNAHSEGYVNVTVEPEPRKNRPPIAIVSPQFQEISLPTTSTVIDGSQSTDDDKIVQYHWEELKGPLREEKISEDTAILKLSKLVPGNYTFRLTVVDSDGATDSTTANLTVNKAVDHHHHHH

SEQ ID NO: 68 - protein, 219 aa, synthetic construct
  REGION 1..219: note = AVR16_K380R
MKYLLPTAAAGLLLLAAQPAMAMGSAGESDQITLPKHEVQLNVYVLLVPPKGEASTYDWQLITHPRDYSGEMEGEHSQILKLSNLTPGLYEYRAVVEGQNAHSEGYVNVTVEPEPRKNRPPIAIVSPQFQEISLPTTSTVIDGSQSTDDDKIVQYHWEELKGPLREEKISEDTAILKLSKLVPGNYTFRLTVVDSDGATDSTTANLTVNKAVDHHHHHH

SEQ ID NO: 69 - DNA, 657 bp, synthetic construct
  source 1..657: mol_type = other DNA
  misc_feature 1..657: note = AVR16_K467Q gene
atgaaatacctgctgccgaccgctgctgctggtctgctgctcctcgctgcccagccggcgatggccatgggctctgcaggcgagtcggatcagattaccctgccgaagcacgaagtacaactgaatgtttatgtgctgctggtaccaccgaaaggggaagcctcgacgtatgactggcagcttattacgcatcctcgcgactacagcggcgagatggaaggagaacattcgcagattctgaaactgtccaatctgacgccgggtctgtatgaatacaaggctgtcgttgaaggtcagaatgcacatagcgaaggctatgttaacgttaccgtggaaccggagccacgcaagaaccgtcctccgatcgccattgtttcaccgcagtttcaggagatttcactgccgaccaccagtaccgttatcgatggttcgcagtcaacggatgacgacaaaatcgttcagtaccactgggaagagctgaaaggccccttacgcgaagagaagatcagcgaagataccgccatcttgaaattatcgcaacttgtgccgggtaactacacgttcagactgacggtggtcgattctgatggcgcaaccgactccaccaccgccaaccttaccgtcaacaaagcggtagaccatcatcatcatcatcat

SEQ ID NO: 70 - protein, 219 aa, synthetic construct
  REGION 1..219: note = AVR16_K467Q
MKYLLPTAAAGLLLLAAQPAMAMGSAGESDQITLPKHEVQLNVYVLLVPPKGEASTYDWQLITHPRDYSGEMEGEHSQILKLSNLTPGLYEYKAVVEGQNAHSEGYVNVTVEPEPRKNRPPIAIVSPQFQEISLPTTSTVIDGSQSTDDDKIVQYHWEELKGPLREEKISEDTAILKLSQLVPGNYTFRLTVVDSDGATDSTTANLTVNKAVDHHHHHH

SEQ ID NO: 71 - protein, 219 aa, synthetic construct
  REGION 1..219: note = AVR16_S482T
MKYLLPTAAAGLLLLAAQPAMAMGSAGESDQITLPKHEVQLNVYVLLVPPKGEASTYDWQLITHPRDYSGEMEGEHSQILKLSNLTPGLYEYKAVVEGQNAHSEGYVNVTVEPEPRKNRPPIAIVSPQFQEISLPTTSTVIDGSQSTDDDKIVQYHWEELKGPLREEKISEDTAILKLSKLVPGNYTFRLTVVDTDGATDSTTANLTVNKAVDHHHHHH

SEQ ID NO: 72 - protein, 219 aa, synthetic construct
  REGION 1..219: note = AVR16_N492D
MKYLLPTAAAGLLLLAAQPAMAMGSAGESDQITLPKHEVQLNVYVLLVPPKGEASTYDWQLITHPRDYSGEMEGEHSQILKLSNLTPGLYEYKAVVEGQNAHSEGYVNVTVEPEPRKNRPPIAIVSPQFQEISLPTTSTVIDGSQSTDDDKIVQYHWEELKGPLREEKISEDTAILKLSKLVPGNYTFRLTVVDSDGATDSTTADLTVNKAVDHHHHHH

SEQ ID NO: 73 - DNA, 30 bp, synthetic construct
  source 1..30: mol_type = other DNA
  misc_feature 1..30: note = Primer S482T-F
ttttggtctcagtggtcgataccgatggcg

SEQ ID NO: 74 - DNA, 28 bp, synthetic construct
  source 1..28: mol_type = other DNA
  misc_feature 1..28: note = Primer S482T-R
ttttggtctcaccaccgtcagtctgaac

SEQ ID NO: 75 - DNA, 32 bp, synthetic construct
  source 1..32: mol_type = other DNA
  misc_feature 1..32: note = Primer V326A-F
ttttggtctcaccgaagcacgaagcacaactg

SEQ ID NO: 76 - DNA, 30 bp, synthetic construct
  source 1..30: mol_type = other DNA
  misc_feature 1..30: note = Primer V326A-R
ttttggtctcatcggcagggtaatctgatc

SEQ ID NO: 77 - DNA, 30 bp, synthetic construct
  source 1..30: mol_type = other DNA
  misc_feature 1..30: note = Primer N492D-F
ttttggtctcacaccgccgatcttaccgtc

SEQ ID NO: 78 - DNA, 29 bp, synthetic construct
  source 1..29: mol_type = other DNA
  misc_feature 1..29: note = Primer N492D-R
ttttggtctcaggtggtggagtcggttgc

SEQ ID NO: 79 - DNA, 33 bp, synthetic construct
  source 1..33: mol_type = other DNA
  misc_feature 1..33: note = Primer K380R-F
ttttggtctcatatgaataccgtgctgtcgttg

SEQ ID NO: 80 - DNA, 28 bp, synthetic construct
  source 1..28: mol_type = other DNA
  misc_feature 1..28: note = Primer K380R-R
ttttggtctcacatacagacccggcgtc

SEQ ID NO: 81 - protein, 219 aa, synthetic construct
  REGION 1..219: note = AVR18
MKYLLPTAAAGLLLLAAQPAMAMGSAGESDQITLPKHEVQLNVYVLLVPPKGEASTYDWQLITHPRDYSGEMEGEHSQILKLSNLTPGLYEYKAVVEGQNAHSEGYVNVTVEPEPRKNRPPIAIVSPQFQEISLPTTSTVIDGSQSTDDDKIVQYHWEELKGPLREEKISEDTAILKLSQLVPGNYTFRLTVVDTDGATDSTTANLTVNKAVDHHHHHH

SEQ ID NO: 82 - DNA, 657 bp, synthetic construct
  source 1..657: mol_type = other DNA
  misc_feature 1..657: note = AVR18 gene
atgaaatacctgctgccgaccgctgctgctggtctgctgctcctcgctgcccagccggcgatggccatgggctctgcaggcgagtcggatcagattaccctgccgaagcacgaagtacaactgaatgtttatgtgctgctggtaccaccgaaaggggaagcctcgacgtatgactggcagcttattacgcatcctcgcgactacagcggcgagatggaaggagaacattcgcagattctgaaactgtccaatctgacgccgggtctgtatgaatacaaggctgtcgttgaaggtcagaatgcacatagcgaaggctatgttaacgttaccgtggaaccggagccacgcaagaaccgtcctccgatcgccattgtttcaccgcagtttcaggagatttcactgccgaccaccagtaccgttatcgatggttcgcagtcaacggatgacgacaaaatcgttcagtaccactgggaagagctgaaaggccccttacgcgaagagaagatcagcgaagataccgccatcttgaaattatcgcaacttgtgccgggtaactacacgttcagactgacggtggtcgataccgatggcgcaaccgactccaccaccgccaaccttaccgtcaacaaagcggtagaccatcatcatcatcatcat

SEQ ID NO: 83 - protein, 219 aa, synthetic construct
  REGION 1..219: note = AVR19a
MKYLLPTAAAGLLLLAAQPAMAMGSAGESDQITLPKHEAQLNVYVLLVPPKGEASTYDWQLITHPRDYSGEMEGEHSQILKLSNLTPGLYEYKAVVEGQNAHSEGYVNVTVEPEPRKNRPPIAIVSPQFQEISLPTTSTVIDGSQSTDDDKIVQYHWEELKGPLREEKISEDTAILKLSQLVPGNYTFRLTVVDTDGATDSTTANLTVNKAVDHHHHHH

SEQ ID NO: 84 - DNA, 657 bp, synthetic construct
  source 1..657: mol_type = other DNA
  misc_feature 1..657: note = AVR19a gene
atgaaatacctgctgccgaccgctgctgctggtctgctgctcctcgctgcccagccggcgatggccatgggctctgcaggcgagtcggatcagattaccctgccgaagcacgaagcacaactgaatgtttatgtgctgctggtaccaccgaaaggggaagcctcgacgtatgactggcagcttattacgcatcctcgcgactacagcggcgagatggaaggagaacattcgcagattctgaaactgtccaatctgacgccgggtctgtatgaatacaaggctgtcgttgaaggtcagaatgcacatagcgaaggctatgttaacgttaccgtggaaccggagccacgcaagaaccgtcctccgatcgccattgtttcaccgcagtttcaggagatttcactgccgaccaccagtaccgttatcgatggttcgcagtcaacggatgacgacaaaatcgttcagtaccactgggaagagctgaaaggccccttacgcgaagagaagatcagcgaagataccgccatcttgaaattatcgcagcttgtgccgggtaactacacgttcagactgacggtggtcgataccgatggcgcaaccgactccaccaccgccaaccttaccgtcaacaaagcggtagaccatcatcatcatcatcat

SEQ ID NO: 85 - protein, 219 aa, synthetic construct
  REGION 1..219: note = AVR19b
MKYLLPTAAAGLLLLAAQPAMAMGSAGESDQITLPKHEVQLNVYVLLVPPKGEASTYDWQLITHPRDYSGEMEGEHSQILKLSNLTPGLYEYKAVVEGQNAHSEGYVNVTVEPEPRKNRPPIAIVSPQFQEISLPTTSTVIDGSQSTDDDKIVQYHWEELKGPLREEKISEDTAILKLSQLVPGNYTFRLTVVDTDGATDSTTADLTVNKAVDHHHHHH

SEQ ID NO: 86 - DNA, 657 bp, synthetic construct
  source 1..657: mol_type = other DNA
  misc_feature 1..657: note = AVR19b gene
atgaaatacctgctgccgaccgctgctgctggtctgctgctcctcgctgcccagccggcgatggccatgggctctgcaggcgagtcggatcagattaccctgccgaagcacgaagtacaactgaatgtttatgtgctgctggtaccaccgaaaggggaagcctcgacgtatgactggcagcttattacgcatcctcgcgactacagcggcgagatggaaggagaacattcgcagattctgaaactgtccaatctgacgccgggtctgtatgaatacaaggctgtcgttgaaggtcagaatgcacatagcgaaggctatgttaacgttaccgtggaaccggagccacgcaagaaccgtcctccgatcgccattgtttcaccgcagtttcaggagatttcactgccgaccaccagtaccgttatcgatggttcgcagtcaacggatgacgacaaaatcgttcagtaccactgggaagagctgaaaggccccttacgcgaagagaagatcagcgaagataccgccatcttgaaattatcgcagcttgtgccgggtaactacacgttcagactgacggtggtcgataccgatggcgcaaccgactccaccaccgccgaccttaccgtcaacaaagcggtagaccatcatcatcatcatcat

SEQ ID NO: 87 - protein, 219 aa, synthetic construct
  REGION 1..219: note = AVR19c
MKYLLPTAAAGLLLLAAQPAMAMGSAGESDQITLPKHEVQLNVYVLLVPPKGEASTYDWQLITHPRDYSGEMEGEHSQILKLSNLTPGLYEYRAVVEGQNAHSEGYVNVTVEPEPRKNRPPIAIVSPQFQEISLPTTSTVIDGSQSTDDDKIVQYHWEELKGPLREEKISEDTAILKLSQLVPGNYTFRLTVVDTDGATDSTTANLTVNKAVDHHHHHH

SEQ ID NO: 88 - protein, 219 aa, synthetic construct
  REGION 1..219: note = AVR20a
MKYLLPTAAAGLLLLAAQPAMAMGSAGESDQITLPKHEAQLNVYVLLVPPKGEASTYDWQLITHPRDYSGEMEGEHSQILKLSNLTPGLYEYKAVVEGQNAHSEGYVNVTVEPEPRKNRPPIAIVSPQFQEISLPTTSTVIDGSQSTDDDKIVQYHWEELKGPLREEKISEDTAILKLSQLVPGNYTFRLTVVDTDGATDSTTADLTVNKAVDHHHHHH

SEQ ID NO: 89 - DNA, 657 bp, synthetic construct
  source 1..657: mol_type = other DNA
  misc_feature 1..657: note = AVR20a gene
atgaaatacctgctgccgaccgctgctgctggtctgctgctcctcgctgcccagccggcgatggccatgggctctgcaggcgagtcggatcagattaccctgccgaagcacgaagcacaactgaatgtttatgtgctgctggtaccaccgaaaggggaagcctcgacgtatgactggcagcttattacgcatcctcgcgactacagcggcgagatggaaggagaacattcgcagattctgaaactgtccaatctgacgccgggtctgtatgaatacaaggctgtcgttgaaggtcagaatgcacatagcgaaggctatgttaacgttaccgtggaaccggagccacgcaagaaccgtcctccgatcgccattgtttcaccgcagtttcaggagatttcactgccgaccaccagtaccgttatcgatggttcgcagtcaacggatgacgacaaaatcgttcagtaccactgggaagagctgaaaggccccttacgcgaagagaagatcagcgaagataccgccatcttgaaattatcgcagcttgtgccgggtaactacacgttcagactgacggtggtcgataccgatggcgcaaccgactccaccaccgccgaccttaccgtcaacaaagcggtagaccatcatcatcatcatcat

SEQ ID NO: 90 - protein, 219 aa, synthetic construct
  REGION 1..219: note = AVR20b
MKYLLPTAAAGLLLLAAQPAMAMGSAGESDQITLPKHEAQLNVYVLLVPPKGEASTYDWQLITHPRDYSGEMEGEHSQILKLSNLTPGLYEYRAVVEGQNAHSEGYVNVTVEPEPRKNRPPIAIVSPQFQEISLPTTSTVIDGSQSTDDDKIVQYHWEELKGPLREEKISEDTAILKLSQLVPGNYTFRLTVVDTDGATDSTTANLTVNKAVDHHHHHH

SEQ ID NO: 91 - protein, 219 aa, synthetic construct
  REGION 1..219: note = AVR20c
MKYLLPTAAAGLLLLAAQPAMAMGSAGESDQITLPKHEVQLNVYVLLVPPKGEASTYDWQLITHPRDYSGEMEGEHSQILKLSNLTPGLYEYRAVVEGQNAHSEGYVNVTVEPEPRKNRPPIAIVSPQFQEISLPTTSTVIDGSQSTDDDKIVQYHWEELKGPLREEKISEDTAILKLSQLVPGNYTFRLTVVDTDGATDSTTADLTVNKAVDHHHHHH

SEQ ID NO: 92 - protein, 219 aa, synthetic construct
  REGION 1..219: note = AVR21
MKYLLPTAAAGLLLLAAQPAMAMGSAGESDQITLPKHEAQLNVYVLLVPPKGEASTYDWQLITHPRDYSGEMEGEHSQILKLSNLTPGLYEYRAVVEGQNAHSEGYVNVTVEPEPRKNRPPIAIVSPQFQEISLPTTSTVIDGSQSTDDDKIVQYHWEELKGPLREEKISEDTAILKLSQLVPGNYTFRLTVVDTDGATDSTTADLTVNKAVDHHHHHH

SEQ ID NO: 93 - DNA, 657 bp, synthetic construct; identical to SEQ ID NO: 35
  source 1..657: mol_type = other DNA
  misc_feature 1..657: note = AVR21 gene

SEQ ID NO: 94 - protein, 1049 aa, Homo sapiens; identical to SEQ ID NO: 1

SEQ ID NO: 95 - protein, 239 aa, synthetic construct; identical to SEQ ID NO: 2
  REGION 1..239: note = Enhanced green fluorescent protein AA

SEQ ID NO: 96 - DNA, 732 bp, synthetic construct; identical to SEQ ID NO: 3
  misc_feature 1..732: note = Enhanced green fluorescent protein DNA
  source 1..732: mol_type = other DNA

SEQ ID NO: 97 - protein, 226 aa, synthetic construct
  REGION 1..226: note = AVR10s AA
MKYLLPTAAAGLLLLAAQPAMAMGSAGESDQITLPKNEVQLNAYVLQEPPKGETSTYDWQLITHPRDYSGEMEGEHSQILKLSNLTPGLYEFKAVVEGQNAHSEGYVNVTVEPEPRKNRPPIAIVSPQFQEISLPTTSTVIDGSQSTDDDKIVQYHWEELKGPLREEKISEDTAILKLSKLVPGNYTFRLTVVDSDGATDSTTANLTVNKAVDHHHHHHCRNDTCG

SEQ ID NO: 98 - DNA, 678 bp, synthetic construct
  misc_feature 1..678: note = AVR10s DNA
  source 1..678: mol_type = other DNA
atgaaatacctgctgccgaccgctgctgctggtctgctgctcctcgctgcccagccggcgatggccatgggctctgcaggcgagtcggatcagattaccctgccgaagaacgaagtacaactgaatgcgtatgtgctgcaggaaccaccgaaaggggaaacctcgacgtatgactggcagcttattacgcatcctcgcgactacagcggcgagatggaaggagaacattcgcagattctgaaactgtccaatctgacgccgggtctgtatgaattcaaggctgtcgttgaaggtcagaatgcacatagcgaaggctatgttaacgttaccgtggaaccggagccacgcaagaaccgtcctccgatcgccattgtttcaccgcagtttcaggagatttcactgccgaccaccagtaccgttatcgatggttcgcagtcaacggatgacgacaaaatcgttcagtaccactgggaagagctgaaaggccccttacgcgaagagaagatcagcgaagataccgccatcttgaaattatcgaaacttgtgccgggtaactacacgttcagactgacggtggtcgattctgatggcgcaaccgactccaccaccgccaaccttaccgtcaacaaagcggtagaccatcatcatcatcatcattgccgcaacgatacctgcgga

SEQ ID NO: 99 - protein, 735 aa, Adeno-Associated virus [sequence omitted]

SEQ ID NO: 100 - protein, 226 aa, synthetic construct
  REGION 1..226: note = AVR11a AA
MKYLLPTAAAGLLLLAAQPAMAMGSAGESDQITLPKNEVQLNVYVLQEPPKGETSTYDWQLITHPRDYSGEMEGEHSQILKLSNLTPGLYEFKAVVEGQNAHSEGYVNVTVEPEPRKNRPPIAIVSPQFQEISLPTTSTVIDGSQSTDDDKIVQYHWEELKGPLREEKISEDTAILKLSKLVPGNYTFRLTVVDSDGATDSTTANLTVNKAVDHHHHHHCRNDTCG

SEQ ID NO: 101 - DNA, 678 bp, synthetic construct
  misc_feature 1..678: note = AVR11a DNA
  source 1..678: mol_type = other DNA
atgaaatacctgctgccgaccgctgctgctggtctgctgctcctcgctgcccagccggcgatggccatgggctctgcaggcgagtcggatcagattaccctgccgaagcacgaagcacaactgaatgtttatgtgctgctggtaccaccgaaaggggaagcctcgacgtatgactggcagcttattacgcatcctcgcgactacagcggcgagatggaaggagaacattcgcagattctgaaactgtccaatctgacgccgggtctgtatgaataccgtgctgtcgttgaaggtcagaatgcacatagcgaaggctatgttaacgttaccgtggaaccggagccacgcaagaaccgtcctccgatcgccattgtttcaccgcagtttcaggagatttcactgccgaccaccagtaccgttatcgatggttcgcagtcaacggatgacgacaaaatcgttcagtaccactgggaagagctgaaaggccccttacgcgaagagaagatcagcgaagataccgccatcttgaaattatcgcagcttgtgccgggtaactacacgttcagactgacggtggtcgataccgatggcgcaaccgactccaccaccgccgatcttaccgtcaacaaagcggtagaccatcatcatcatcatcattgccgcaacgatacctgcgga

SEQ ID NO: 102 - protein, 226 aa, synthetic construct
  REGION 1..226: note = AVR21 AA
MKYLLPTAAAGLLLLAAQPAMAMGSAGESDQITLPKHEAQLNVYVLLVPPKGEASTYDWQLITHPRDYSGEMEGEHSQILKLSNLTPGLYEYRAVVEGQNAHSEGYVNVTVEPEPRKNRPPIAIVSPQFQEISLPTTSTVIDGSQSTDDDKIVQYHWEELKGPLREEKISEDTAILKLSQLVPGNYTFRLTVVDTDGATDSTTADLTVNKAVDHHHHHHCRNDTCG

SEQ ID NO: 103 - DNA, 678 bp, synthetic construct; identical to SEQ ID NO: 101
  misc_feature 1..678: note = AVR21 DNA
  source 1..678: mol_type = other DNA